European Patent Application EP 4 389 889 A2, published June 26, 2024. Title: Compositions and methods for editing RNA. Applicant: Oregon Health & Science University. Application EP, filed October 9, 2018. The sequence listing filed with the application follows.

SEQUENCE LISTING (72 sequences)

SEQ ID NO: 1 - DNA, 34 bp, synthetic construct
  misc_feature 1..34: note = mMecp2 E1 Fwd EcoRI primer
  source 1..34: mol_type = other DNA
gcgcgaattccaccatggccgccgctgccgccac

SEQ ID NO: 2 - DNA, 33 bp, synthetic construct
  misc_feature 1..33: note = mMecp2 E1 Rev KpnI no stop codon primer
  source 1..33: mol_type = other DNA
gcgcgggtaccgctaactctctcggtcacgggc

SEQ ID NO: 3 - DNA, 35 bp, synthetic construct
  misc_feature 1..35: note = mMecp2 W104X mut primer Fwd primer
  source 1..35: mol_type = other DNA
caccttgcctgaaggttagacacgaaagcttaaac

SEQ ID NO: 4 - DNA, 35 bp, synthetic construct
  misc_feature 1..35: note = mMecp2 W104X mut primer Rev primer
  source 1..35: mol_type = other DNA
gtttaagctttcgtgtctaaccttcaggcaaggtg

SEQ ID NO: 5 - DNA, 33 bp, synthetic construct
  misc_feature 1..33: note = mMecp2 R106Q mut primer Fwd primer
  source 1..33: mol_type = other DNA
cctgaaggttggacacaaaagcttaaacaaagg

SEQ ID NO: 6 - DNA, 33 bp, synthetic construct
  misc_feature 1..33: note = mMecp2 R106Q mut primer Rev primer
  source 1..33: mol_type = other DNA
cctttgtttaagcttttgtgtccaaccttcagg

SEQ ID NO: 7 - DNA, 27 bp, synthetic construct
  misc_feature 1..27: note = mMecp2 R306H mut primer Fwd primer
  source 1..27: mol_type = other DNA
cccatcaagaagcacaagacccgggag

SEQ ID NO: 8 - DNA, 27 bp, synthetic construct
  misc_feature 1..27: note = mMecp2 R306H mut primer Rev primer
  source 1..27: mol_type = other DNA
ctcccgggtcttgtgcttcttgatggg

SEQ ID NO: 9 - DNA, 79 bp, synthetic construct
  misc_feature 1..79: note = Editase EcoRI Kozak HA Fwd primer
  source 1..79: mol_type = other DNA
gaattcgccaccatggtgtacccctatgacgtgcctgactacgccagcggctatccatacgatgtccccgattatgctt

SEQ ID NO: 10 - DNA, 76 bp, synthetic construct
  misc_feature 1..76: note = Editase HA BspEI Rev primer
  source 1..76: mol_type = other DNA
ccggaagcataatcggggacatcgtatggatagccgcaggcgtagtcaggcacgtcataggggtaccatggtggcg

SEQ ID NO: 11 - DNA, 22 bp, synthetic construct
  misc_feature 1..22: note = EGFP F2 primer
  source 1..22: mol_type = other DNA
caccatcttcttcaaggacgac

SEQ ID NO: 12 - DNA, 32 bp, synthetic construct
  misc_feature 1..32: note = SV40 3xNLS Rev primer
  source 1..32: mol_type = other DNA
gacaatccggaggtggatcctacctttctctt

SEQ ID NO: 13 - DNA, 27 bp, synthetic construct
  misc_feature 1..27: note = hDD E488Q Fwd primer
  source 1..27: mol_type = other DNA
aatagagtctggtcaggggacgattcc

SEQ ID NO: 14 - DNA, 27 bp, synthetic construct
  misc_feature 1..27: note = hDD E488Q Rev primer
  source 1..27: mol_type = other DNA
ggaatcgtcccctgaccagactctatt

SEQ ID NO: 15 - DNA, 86 bp, synthetic construct
  misc_feature 1..86: note = mMecp2 W104X 2xBoxB Guide Fwd
  source 1..86: mol_type = other DNA
caccgtcctttgtttggccctgaaaaagggccctttcgtgtccaaccttcaggcaaggggccctgaaaaagggccggtcatcatac

SEQ ID NO: 16 - DNA, 86 bp, synthetic construct
  misc_feature 1..86: note = mMecp2 W104X 2xBoxB Guide Rev
  source 1..86: mol_type = other DNA
aaaagtatgatgaccggccctttttcagggccccttgcctgaaggttggacacgaaagggccctttttcagggccaaacaaaggac

SEQ ID NO: 17 - DNA, 88 bp, synthetic construct
  misc_feature 1..88: note = mMecp2 R106Q 2xBoxB Guide Fwd
  source 1..88: mol_type = other DNA
caccgcagacttcctggccctgaaaaagggcctttaagctttcgtgtccaaccttcaggcaggccctgaaaaagggcctggggtcatc

SEQ ID NO: 18 - DNA, 88 bp, synthetic construct
  misc_feature 1..88: note = mMecp2 R106Q 2xBoxB Guide Rev
  source 1..88: mol_type = other DNA
aaaagatgaccccaggccctttttcagggcctgcctgaaggttggacacgaaagcttaaaggccctttttcagggccaggaagtctgc

SEQ ID NO: 19 - DNA, 89 bp, synthetic construct
  misc_feature 1..89: note = mMecp2 R306H 2xBoxB Guide Fwd
  source 1..89: mol_type = other DNA
caccgatgctgaccgtggccctgaaaaagggccccgggtcttgcgcttcttgatgggagcaggccctgaaaaagggcctctcatgcaca

SEQ ID NO: 20 - DNA, 90 bp, synthetic construct
  misc_feature 1..90: note = mMecp2 R306H 2xBoxB Guide Rev
  source 1..90: mol_type = other DNA
aaaatgtgcatgagaggccctttttcagggcctgctccccatcaagaagcgcaagacccggggccctttttcagggccacggtcagcatc

SEQ ID NO: 21 - DNA, 89 bp, synthetic construct
  misc_feature 1..89: note = mMecp2 R106Q Off-target mismatch 2xBoxB Guide Fwd
  source 1..89: mol_type = other DNA
caccgcagacttcctggccctgaaaaagggcctttaagctttccgggtccaaccttcaggcaggccctgaaaaagggcctggggtcatc

SEQ ID NO: 22 - DNA, 88 bp, synthetic construct
  misc_feature 1..88: note = mMecp2 R106Q Off-target mismatch 2xBoxB Guide Rev
  source 1..88: mol_type = other DNA
aaaagatgaccccaggccctttttcagggcctgcctgaaggttggacccgaaagcttaaaggccctttttcagggccaggaagtctgc

SEQ ID NO: 23 - DNA, 25 bp, synthetic construct
  misc_feature 1..25: note = CMV-mMecp2 ATG Fwd primer
  source 1..25: mol_type = other DNA
tcaagcttcgaattccaccatggcc

SEQ ID NO: 24 - DNA, 21 bp, synthetic construct
  misc_feature 1..21: note = GFP-N3 Linker Rev primer
  source 1..21: mol_type = other DNA
ccttgctcaccatggtggcga

SEQ ID NO: 25 - DNA, 20 bp, synthetic construct
  misc_feature 1..20: note = mMecp2 -14 mMecp2 ATG Fwd primer
  source 1..20: mol_type = other DNA
aacccgtccggaaaatggcc

SEQ ID NO: 26 - DNA, 29 bp, synthetic construct
  misc_feature 1..29: note = mMecp2-3'UTR+92 Rev primer
  source 1..29: mol_type = other DNA
ggaagctttgtcagagccctacccataag

SEQ ID NO: 27 - DNA, 21 bp, synthetic construct
  misc_feature 1..21: note = mMecp2 554 Rev primer
  source 1..21: mol_type = other DNA
ctcctggaggggctccctctc

SEQ ID NO: 28 - DNA, 22 bp, synthetic construct
  misc_feature 1..22: note = mMecp2 914 Rev primer
  source 1..22: mol_type = other DNA
gaccgtatggaagactccttca

SEQ ID NO: 29 - DNA, 18 bp, synthetic construct
  misc_feature 1..18: note = mMecp2 1122 Rev primer
  source 1..18: mol_type = other DNA
actgctgctgcgcccctt

SEQ ID NO: 30 - DNA, 31 bp, synthetic construct
  misc_feature 1..31: note = hU6 AflII Fwd primer
  source 1..31: mol_type = other DNA
gtgtcttaaggagggcctatttcccatgatt

SEQ ID NO: 31 - DNA, 31 bp, synthetic construct
  misc_feature 1..31: note = hU6 MfeI Fwd primer
  source 1..31: mol_type = other DNA
gtgtcaattggagggcctatttcccatgatt

SEQ ID NO: 32 - DNA, 31 bp, synthetic construct
  misc_feature 1..31: note = hU6 NheI Fwd primer
  source 1..31: mol_type = other DNA
gtgtgctagcgagggcctatttcccatgatt

SEQ ID NO: 33 - DNA, 31 bp, synthetic construct
  misc_feature 1..31: note = hU6 SacI Fwd primer
  source 1..31: mol_type = other DNA
gtgtgagctcgagggcctatttcccatgatt

SEQ ID NO: 34 - DNA, 28 bp, synthetic construct
  misc_feature 1..28: note = hU6 SpeI Fwd primer
  source 1..28: mol_type = other DNA
gtgtactagtgagggcctatttcccatg

SEQ ID NO: 35 - DNA, 28 bp, synthetic construct
  misc_feature 1..28: note = hU6 (m) NdeI Fwd primer
  source 1..28: mol_type = other DNA
gtgtcatatgcttaccgtaacttgaaag

SEQ ID NO: 36 - DNA, 32 bp, synthetic construct
  misc_feature 1..32: note = R106QgV2 AflII Rev primer
  source 1..32: mol_type = other DNA
atatcttaagaaaaaagatgaccccaggccct

SEQ ID NO: 37 - DNA, 32 bp, synthetic construct
  misc_feature 1..32: note = R106QgV2 ApaI Rev primer
  source 1..32: mol_type = other DNA
cacagggcccaaaaaagatgaccccaggccct

SEQ ID NO: 38 - DNA, 32 bp, synthetic construct
  misc_feature 1..32: note = R106QgV2 MfeI Rev primer
  source 1..32: mol_type = other DNA
atatcaattgaaaaaagatgaccccaggccct

SEQ ID NO: 39 - DNA, 32 bp, synthetic construct
  misc_feature 1..32: note = R106QgV2 SacI Rev primer
  source 1..32: mol_type = other DNA
atatgagctcaaaaaagatgaccccaggccct

SEQ ID NO: 40 - DNA, 32 bp, synthetic construct
  misc_feature 1..32: note = R106QgV2 SpeI Rev primer
  source 1..32: mol_type = other DNA
atatactagtaaaaaagatgaccccaggccct

SEQ ID NO: 41 - DNA, 44 bp, synthetic construct
  misc_feature 1..44: note = R106QgV2 (+2)ApaI Rev primer
  source 1..44: mol_type = other DNA
gcgcgggcccttcgaagctagcaaaaaagatgaccccaggccct

SEQ ID NO: 42 - DNA, 31 bp, synthetic construct
  misc_feature 1..31: note = 2xHA Editase Fwd NcoI Kozak primer
  source 1..31: mol_type = other DNA
attcgccaccatggtgtacccctatgacgtg

SEQ ID NO: 43 - DNA, 30 bp, synthetic construct
  misc_feature 1..30: note = Editase EcoRI Rev primer
  source 1..30: mol_type = other DNA
gcgcgaattctcaatggtgatggtgatggt

SEQ ID NO: 44 - protein, 50 aa, synthetic construct
  REGION 1..50: note = linker
  VARIANT 6..10: note = amino acids 6-10 are GGGGS or absent
  VARIANT 11..15: note = amino acids 11-15 are GGGGS or absent
  VARIANT 16..20: note = amino acids 16-20 are GGGGS or absent
  VARIANT 21..25: note = amino acids 21-25 are GGGGS or absent
  VARIANT 26..30: note = amino acids 26-30 are GGGGS or absent
  VARIANT 31..35: note = amino acids 31-35 are GGGGS or absent
  VARIANT 36..40: note = amino acids 36-40 are GGGGS or absent
  VARIANT 41..45: note = amino acids 41-45 are GGGGS or absent
  VARIANT 46..50: note = amino acids 46-50 are GGGGS or absent
GGGGSXXXXXXXXXXXXXXXXXXXXXXXXXXXXXXXXXXXXXXXXXXXXX

SEQ ID NO: 45 - protein, 15 aa, synthetic construct
  REGION 1..15: note = linker
GGGGSGGGGSGGGGS

SEQ ID NO: 46 - protein, 22 aa, synthetic construct
  REGION 1..22: note = lambda N peptide
MNARTRRRERRAEKQAQWKAAN

SEQ ID NO: 47 - protein, 7 aa, synthetic construct
  REGION 1..7: note = SV40 Large T-antigen NLS
PKKKRKV

SEQ ID NO: 48 - RNA, 15 nt, synthetic construct
  misc_feature 1..15: note = BoxB sequence
  source 1..15: mol_type = other RNA
gccctgaaaaagggc

SEQ ID NO: 49 - RNA, 17 nt, synthetic construct
  misc_feature 1..17: note = BoxB sequence
  source 1..17: mol_type = other RNA
ggccctgaaaaagggcc

SEQ ID NO: 50 - DNA, 20 bp, synthetic construct
  misc_feature 1..20: note = Mecp2-R106Q Fwd primer
  source 1..20: mol_type = other DNA
ggacctatgtatgatgaccc

SEQ ID NO: 51 - DNA, 20 bp, synthetic construct
  misc_feature 1..20: note = Mecp2-R106Q Rev primer
  source 1..20: mol_type = other DNA
ggtcattgggctagactgaa

SEQ ID NO: 52 - DNA, 30 bp, synthetic construct
  misc_feature 1..30: note = target sequence
  source 1..30: mol_type = other DNA
ttgcctgaaggttggacacaaaagcttaaa

SEQ ID NO: 53 - protein, 10 aa, synthetic construct
  REGION 1..10: note = target sequence
LPEGWTQKLK

SEQ ID NO: 54 - protein, 9 aa, synthetic construct
  REGION 1..9: note = c-myc NLS
PAAKRVKLD

SEQ ID NO: 55 - protein, 403 aa, synthetic construct
  REGION 1..403: note = deaminase domain of human ADAR2
LHLDQTPSRQPIPSEGLQLHLPQVLADAVSRLVLGKFGDLTDNFSSPHARRKVLAGVVMTTGTDVKDAKVISVSTGTKCINGEYMSDRGLALNDCHAEIISRRSLLRFLYTQLELYLNNKDDQKRSIFQKSERGGFRLKENVQFHLYISTSPCGDARIFSPHEPILEEPADRHPNRKARGQLRTKIESGEGTIPVRSNASIQTWDGVLQGERLLTMSCSDKIARWNVVGIQGSLLSIFVEPIYFSSIILGSLYHGDHLSRAMYQRISNIEDLPPLYTLNKPLLSGISNAEARQPGKAPNFSVNWTVGDSAIEVINATTGKDELGRASRLCKHALYCRWMRVHGKVPSHLLRSKITKPNVYHESKLAAKEYQAAKARLFTAFIKAGLGAWVEKPTEQDQFSLTP

SEQ ID NO: 56 - protein, 486 aa, Homo sapiens
MVAGMLGLREEKSEDQDLQGLKDKPLKFKKVKKDKKEEKEGKHEPVQPSAHHSAEPAEAGKAETSEGSGSAPAVPEASASPKQRRSIIRDRGPMYDDPTLPEGWTRKLKQRKSGRSAGKYDVYLINPQGKAFRSKVELIAYFEKVGDTSLDPNDFDFTVTGRGSPSRREQKPPKKPKSPKAPGTGRGRGRPKGSGTTRPKAATSEGVQVKRVLEKSPGKLLVKMPFQTSPGGKAEGGGATTSTQVMVIKRPGRKRKAEADPQAIPKKRGRKPGSVVAAAAAEAKKKAVKESSIRSVQETVLPIKKRKTRETVSIEVKEVVKPLLVSTLGEKSGKGLKTCKSPGRKSKESSPKGRSSSASSPPKKEHHHHHHHSESPKAPVPLLPPLPPPPPEPESSEDPTSPPEPQDLSSSVCKEEKMPRGGSLESDGCPKEPAKTQPAVATAATAAEKYKHRGEGERKDIVSSSMPRPNREEPVDSRTPVTERVS

SEQ ID NO: 57 - DNA, 1461 bp, Homo sapiens
  source 1..1461: mol_type = other DNA
atggtagctgggatgttagggctcagggaagaaaagtcagaagaccaggacctccagggcctcaaggacaaacccctcaagtttaaaaaggtgaagaaagataagaaagaagagaaagagggcaagcatgagcccgtgcagccatcagcccaccactctgctgagcccgcagaggcaggcaaagcagagacatcagaagggtcaggctccgccccggctgtgccggaagcttctgcctcccccaaacagcggcgctccatcatccgtgaccggggacccatgtatgatgaccccaccctgcctgaaggctggacacggaagcttaagcaaaggaaatctggccgctctgctgggaagtatgatgtgtatttgatcaatccccagggaaaagcctttcgctctaaagtggagttgattgcgtacttcgaaaaggtaggcgacacatccctggaccctaatgattttgacttcacggtaactgggagagggagcccctcccggcgagagcagaaaccacctaagaagcccaaatctcccaaagctccaggaactggcagaggccggggacgccccaaagggagcggcaccacgagacccaaggcggccacgtcagagggtgtgcaggtgaaaagggtcctggagaaaagtcctgggaagctccttgtcaagatgccttttcaaacttcgccagggggcaaggctgaggggggtggggccaccacatccacccaggtcatggtgatcaaacgccccggcaggaagcgaaaagctgaggccgaccctcaggccattcccaagaaacggggccgaaagccggggagtgtggtggcagccgctgccgccgaggccaaaaagaaagccgtgaaggagtcttctatccgatctgtgcaggagaccgtactccccatcaagaagcgcaagacccgggagacggtcagcatcgaggtcaaggaagtggtgaagcccctgctggtgtccaccctcggtgagaagagcgggaaaggactgaagacctgtaagagccctgggcggaaaagcaaggagagcagccccaaggggcgcagcagcagcgcctcctcaccccccaagaaggagcaccaccaccatcaccaccactcagagtccccaaaggcccccgtgccactgctcccacccctgcccccacctccacctgagcccgagagctccgaggaccccaccagcccccctgagccccaggacttgagcagcagcgtctgcaaagaggagaagatgcccagaggaggctcactggagagcgacggctgccccaaggagccagctaagactcagcccgcggttgccaccgccgccacggccgcagaaaagtacaaacaccgaggggagggagagcgcaaagacattgtttcatcctccatgccaaggccaaacagagaggagcctgtggacagccggacgcccgtgaccgagagagttagctga

SEQ ID NO: 58-59 - skipped (2 entries)

SEQ ID NO: 60 - protein, 16 aa, synthetic construct
  REGION 1..16: note = nucleopplasmin NLS
KRPAATKKAGQAKKKK

SEQ ID NO: 61 - DNA, 30 bp, synthetic construct
  misc_feature 1..30: note = hADAR2 3xFlag Fwd primer
  source 1..30: mol_type = other DNA
tggtggaattcgccaccatggactacaagg

SEQ ID NO: 62 - DNA, 28 bp, synthetic construct
  misc_feature 1..28: note = hADAR2 Rev primer
  source 1..28: mol_type = other DNA
tcgagcggccgctcaatggtgatggtga

SEQ ID NO: 63 - DNA, 60 bp, synthetic construct
  misc_feature 1..60: note = mMecp2 W104X Internal loop Guide Fwd
  source 1..60: mol_type = other DNA
caccgacttcctttgttattgctttcgggtccaaccttcaggcatcctggggtcatcata

SEQ ID NO: 64 - DNA, 60 bp, synthetic construct
  misc_feature 1..60: note = mMecp2 W104X Internal loop Guide Rev
  source 1..60: mol_type = other DNA
aaaatatgatgaccccaggatgcctgaaggttggacccgaaagcaataacaaaggaagtc

SEQ ID NO: 65 - DNA, 92 bp, synthetic construct
  misc_feature 1..92: note = mMecp2 W104X GluA2 Guide Fwd
  source 1..92: mol_type = other DNA
caccgtggaatagtataacaatatgctaaatgttgttatagtatcccactcgtgtccaaccttcatctagagggccctgaagagggcccttt

SEQ ID NO: 66 - DNA, 92 bp, synthetic construct
  misc_feature 1..92: note = mMecp2 W104X GluA2 Guide Rev
  source 1..92: mol_type = other DNA
aaaaaaagggccctcttcagggccctctagatgaaggttggacacgagtgggatactataacaacatttagcatattgttatactattccac

SEQ ID NO: 67 - protein, 24 aa, synthetic construct
  REGION 1..24: note = NLS
DPKKKRKVDPKKKRKVDPKKKRKV

SEQ ID NO: 68 - protein, 440 aa, synthetic construct
  REGION 1..440: note = fusion protein
MNARTRRRERRAEKQAQWKAANGGGGSGGGGSGGGGSLHLDQTPSRQPIPSEGLQLHLPQVLADAVSRLVLGKFGDLTDNFSSPHARRKVLAGVVMTTGTDVKDAKVISVSTGTKCINGEYMSDRGLALNDCHAEIISRRSLLRFLYTQLELYLNNKDDQKRSIFQKSERGGFRLKENVQFHLYISTSPCGDARIFSPHEPILEEPADRHPNRKARGQLRTKIESGEGTIPVRSNASIQTWDGVLQGERLLTMSCSDKIARWNVVGIQGSLLSIFVEPIYFSSIILGSLYHGDHLSRAMYQRISNIEDLPPLYTLNKPLLSGISNAEARQPGKAPNFSVNWTVGDSAIEVINATTGKDELGRASRLCKHALYCRWMRVHGKVPSHLLRSKITKPNVYHESKLAAKEYQAAKARLFTAFIKAGLGAWVEKPTEQDQFSLTP

SEQ ID NO: 69 - protein, 464 aa, synthetic construct
  REGION 1..464: note = fusion protein
DPKKKRKVDPKKKRKVDPKKKRKVMNARTRRRERRAEKQAQWKAANGGGGSGGGGSGGGGSLHLDQTPSRQPIPSEGLQLHLPQVLADAVSRLVLGKFGDLTDNFSSPHARRKVLAGVVMTTGTDVKDAKVISVSTGTKCINGEYMSDRGLALNDCHAEIISRRSLLRFLYTQLELYLNNKDDQKRSIFQKSERGGFRLKENVQFHLYISTSPCGDARIFSPHEPILEEPADRHPNRKARGQLRTKIESGEGTIPVRSNASIQTWDGVLQGERLLTMSCSDKIARWNVVGIQGSLLSIFVEPIYFSSIILGSLYHGDHLSRAMYQRISNIEDLPPLYTLNKPLLSGISNAEARQPGKAPNFSVNWTVGDSAIEVINATTGKDELGRASRLCKHALYCRWMRVHGKVPSHLLRSKITKPNVYHESKLAAKEYQAAKARLFTAFIKAGLGAWVEKPTEQDQFSLTP

SEQ ID NO: 70 - RNA, 45 nt, synthetic construct
  misc_feature 1..45: note = R/G binding site
  source 1..45: mol_type = other RNA
gtggaatagtataacaatatgctaaatgttgttatagtatcccac

SEQ ID NO: 71 - protein, 403 aa, synthetic construct
  REGION 1..403: note = demainase domain of human ADAR2 E488Q
LHLDQTPSRQPIPSEGLQLHLPQVLADAVSRLVLGKFGDLTDNFSSPHARRKVLAGVVMTTGTDVKDAKVISVSTGTKCINGEYMSDRGLALNDCHAEIISRRSLLRFLYTQLELYLNNKDDQKRSIFQKSERGGFRLKENVQFHLYISTSPCGDARIFSPHEPILEEPADRHPNRKARGQLRTKIESGQGTIPVRSNASIQTWDGVLQGERLLTMSCSDKIARWNVVGIQGSLLSIFVEPIYFSSIILGSLYHGDHLSRAMYQRISNIEDLPPLYTLNKPLLSGISNAEARQPGKAPNFSVNWTVGDSAIEVINATTGKDELGRASRLCKHALYCRWMRVHGKVPSHLLRSKITKPNVYHESKLAAKEYQAAKARLFTAFIKAGLGAWVEKPTEQDQFSLTP

SEQ ID NO: 72 - protein, 1226 aa, Homo sapiens
MNPRQGYSLSGYYTHPFQGYEHRQLRYQQPGPGSSPSSFLLKQIEFLKGQLPEAPVIGKQTPSLPPSLPGLRPRFPVLLASSTRGRQVDIRGVPRGVHLRSQGLQRGFQHPSPRGRSLPQRGVDCLSSHFQELSIYQDQEQRILKFLEELGEGKATTAHDLSGKLGTPKKEINRVLYSLAKKGKLQKEAGTPPLWKIAVSTQAWNQHSGVVRPDGHSQGAPNSDPSLEPEDRNSTSVSEDLLEPFIAVSAQAWNQHSGVVRPDSHSQGSPNSDPGLEPEDSNSTSALEDPLEFLDMAEIKEKICDYLFNVSDSSALNLAKNIGLTKARDINAVLIDMERQGDVYRQGTTPPIWHLTDKKRERMQIKRNTNSVPETAPAAIPETKRNAEFLTCNIPTSNASNNMVTTEKVENGQEPVIKLENRQEARPEPARLKPPVHYNGPSKAGYVDFENGQWATDDIPDDLNSIRAAPGEFRAIMEMPSFYSHGLPRCSPYKKLTECQLKNPISGLLEYAQFASQTCEFNMIEQSGPPHEPRFKFQVVINGREFPPAEAGSKKVAKQDAAMKAMTILLEEAKAKDSGKSEESSHYSTEKESEKTAESQTPTPSATSFFSGKSPVTTLLECMHKLGNSCEFRLLSKEGPAHEPKFQYCVAVGAQTFPSVSAPSKKVAKQMAAEEAMKALHGEATNSMASDNQPEGMISESLDNLESMMPNKVRKIGELVRYLNTNPVGGLLEYARSHGFAAEFKLVDQSGPPHEPKFVYQAKVGGRWFPAVCAHSKKQGKQEAADAALRVLIGENEKAERMGFTEVTPVTGASLRRTMLLLSRSPEAQPKTLPLTGSTFHDQIAMLSHRCFNTLTNSFQPSLLGRKILAAIIMKKDSEDMGVVVSLGTGNRCVKGDSLSLKGETVNDCHAEIISRRGFIRFLYSELMKYNSQTAKDSIFEPAKGGEKLQIKKTVSFHLYISTAPCGDGALFDKSCSDRAMESTESRHYPVFENPKQGKLRTKVENGEGTIPVESSDIVPTWDGIRLGERLRTMSCSDKILRWNVLGLQGALLTHFLQPIYLKSVTLGYLFSQGHLTRAICCRVTRDGSAFEDGLRHPFIVNHPKVGRVSIYDSKRQSGKTKETSVNWCLADGYDLEILDGTRGTVDGPRNELSRVSKKNIFLLFKKLCSFRYRRDLLRLSYGEAKKAARDYETAKNYFKKGLKDMGYGNWISKPQEEKNFYLCPV